European Patent Application EP 4 122 481 A1, published January 25, 2023. Title: METHOD AND DRUG FOR TREATING HUNTINGTON'S DISEASE. Applicant: TALENGEN INTERNATIONAL LIMITED. Application PCT/CN2021/082725. The sequence listing filed with the application follows.

SEQUENCE LISTING (14 sequences)

SEQ ID NO: 1 - DNA, 2376 bp, Artificial sequence
  nucleotide sequence of the natural plasminogen(Glu-PLG,Glu-plasminogen)without the signal peptide
gagcctctggatgactatgtgaatacccagggggcttcactgttcagtgtcactaagaagcagctgggagcaggaagtatagaagaatgtgcagcaaaatgtgaggaggacgaagaattcacctgcagggcattccaatatcacagtaaagagcaacaatgtgtgataatggctgaaaacaggaagtcctccataatcattaggatgagagatgtagttttatttgaaaagaaagtgtatctctcagagtgcaagactgggaatggaaagaactacagagggacgatgtccaaaacaaaaaatggcatcacctgtcaaaaatggagttccacttctccccacagacctagattctcacctgctacacacccctcagagggactggaggagaactactgcaggaatccagacaacgatccgcaggggccctggtgctatactactgatccagaaaagagatatgactactgcgacattcttgagtgtgaagaggaatgtatgcattgcagtggagaaaactatgacggcaaaatttccaagaccatgtctggactggaatgccaggcctgggactctcagagcccacacgctcatggatacattccttccaaatttccaaacaagaacctgaagaagaattactgtcgtaaccccgatagggagctgcggccttggtgtttcaccaccgaccccaacaagcgctgggaactttgtgacatcccccgctgcacaacacctccaccatcttctggtcccacctaccagtgtctgaagggaacaggtgaaaactatcgcgggaatgtggctgttaccgtgtccgggcacacctgtcagcactggagtgcacagacccctcacacacataacaggacaccagaaaacttcccctgcaaaaatttggatgaaaactactgccgcaatcctgacggaaaaagggccccatggtgccatacaaccaacagccaagtgcggtgggagtactgtaagataccgtcctgtgactcctccccagtatccacggaacaattggctcccacagcaccacctgagctaacccctgtggtccaggactgctaccatggtgatggacagagctaccgaggcacatcctccaccaccaccacaggaaagaagtgtcagtcttggtcatctatgacaccacaccggcaccagaagaccccagaaaactacccaaatgctggcctgacaatgaactactgcaggaatccagatgccgataaaggcccctggtgttttaccacagaccccagcgtcaggtgggagtactgcaacctgaaaaaatgctcaggaacagaagcgagtgttgtagcacctccgcctgttgtcctgcttccagatgtagagactccttccgaagaagactgtatgtttgggaatgggaaaggataccgaggcaagagggcgaccactgttactgggacgccatgccaggactgggctgcccaggagccccatagacacagcattttcactccagagacaaatccacgggcgggtctggaaaaaaattactgccgtaaccctgatggtgatgtaggtggtccctggtgctacacgacaaatccaagaaaactttacgactactgtgatgtccctcagtgtgcggccccttcatttgattgtgggaagcctcaagtggagccgaagaaatgtcctggaagggttgtaggggggtgtgtggcccacccacattcctggccctggcaagtcagtcttagaacaaggtttggaatgcacttctgtggaggcaccttgatatccccagagtgggtgttgactgctgcccactgcttggagaagtccccaaggccttcatcctacaaggtcatcctgggtgcacaccaagaagtgaatctcgaaccgcatgttcaggaaatagaagtgtctaggctgttcttggagcccacacgaaaagatattgccttgctaaagctaagcagtcctgccgtcatcactgacaaagtaatcccagcttgtctgccatccccaaattatgtggtcgctgaccggaccgaatgtttcatcactggctggggagaaacccaaggtacttttggagctggccttctcaaggaagcccagctccctgtgattgagaataaagtgtgcaatcgctatgagtttctgaatggaagagtccaatccaccgaactctgtgctgggcatttggccggaggcactgacagttgccagggtgacagtggaggtcctctggtttgcttcgagaaggacaaatacattttacaaggagtcacttcttggggtcttggctgtgcacgccccaataagcctggtgtctatgttcgtgtttcaaggtttgttacttggattgagggagtgatgagaaataattaa

SEQ ID NO: 2 - protein, 791 aa, Artificial sequence
  amino acid sequence of the natural plasminogen (Glu-PLG,Glu-plasminogen) without the signal peptide
EPLDDYVNTQGASLFSVTKKQLGAGSIEECAAKCEEDEEFTCRAFQYHSKEQQCVIMAENRKSSIIIRMRDVVLFEKKVYLSECKTGNGKNYRGTMSKTKNGITCQKWSSTSPHRPRFSPATHPSEGLEENYCRNPDNDPQGPWCYTTDPEKRYDYCDILECEEECMHCSGENYDGKISKTMSGLECQAWDSQSPHAHGYIPSKFPNKNLKKNYCRNPDRELRPWCFTTDPNKRWELCDIPRCTTPPPSSGPTYQCLKGTGENYRGNVAVTVSGHTCQHWSAQTPHTHNRTPENFPCKNLDENYCRNPDGKRAPWCHTTNSQVRWEYCKIPSCDSSPVSTEQLAPTAPPELTPVVQDCYHGDGQSYRGTSSTTTTGKKCQSWSSMTPHRHQKTPENYPNAGLTMNYCRNPDADKGPWCFTTDPSVRWEYCNLKKCSGTEASVVAPPPVVLLPDVETPSEEDCMFGNGKGYRGKRATTVTGTPCQDWAAQEPHRHSIFTPETNPRAGLEKNYCRNPDGDVGGPWCYTTNPRKLYDYCDVPQCAAPSFDCGKPQVEPKKCPGRVVGGCVAHPHSWPWQVSLRTRFGMHFCGGTLISPEWVLTAAHCLEKSPRPSSYKVILGAHQEVNLEPHVQEIEVSRLFLEPTRKDIALLKLSSPAVITDKVIPACLPSPNYVVADRTECFITGWGETQGTFGAGLLKEAQLPVIENKVCNRYEFLNGRVQSTELCAGHLAGGTDSCQGDSGGPLVCFEKDKYILQGVTSWGLGCARPNKPGVYVRVSRFVTWIEGVMRNN

SEQ ID NO: 3 - DNA, 2433 bp, Artificial sequence
  nucleotide sequence of the natural plasminogen(from swiss prot)with the signal peptide
atggaacataaggaagtggttcttctacttcttttatttctgaaatcaggtcaaggagagcctctggatgactatgtgaatacccagggggcttcactgttcagtgtcactaagaagcagctgggagcaggaagtatagaagaatgtgcagcaaaatgtgaggaggacgaagaattcacctgcagggcattccaatatcacagtaaagagcaacaatgtgtgataatggctgaaaacaggaagtcctccataatcattaggatgagagatgtagttttatttgaaaagaaagtgtatctctcagagtgcaagactgggaatggaaagaactacagagggacgatgtccaaaacaaaaaatggcatcacctgtcaaaaatggagttccacttctccccacagacctagattctcacctgctacacacccctcagagggactggaggagaactactgcaggaatccagacaacgatccgcaggggccctggtgctatactactgatccagaaaagagatatgactactgcgacattcttgagtgtgaagaggaatgtatgcattgcagtggagaaaactatgacggcaaaatttccaagaccatgtctggactggaatgccaggcctgggactctcagagcccacacgctcatggatacattccttccaaatttccaaacaagaacctgaagaagaattactgtcgtaaccccgatagggagctgcggccttggtgtttcaccaccgaccccaacaagcgctgggaactttgtgacatcccccgctgcacaacacctccaccatcttctggtcccacctaccagtgtctgaagggaacaggtgaaaactatcgcgggaatgtggctgttaccgtgtccgggcacacctgtcagcactggagtgcacagacccctcacacacataacaggacaccagaaaacttcccctgcaaaaatttggatgaaaactactgccgcaatcctgacggaaaaagggccccatggtgccatacaaccaacagccaagtgcggtgggagtactgtaagataccgtcctgtgactcctccccagtatccacggaacaattggctcccacagcaccacctgagctaacccctgtggtccaggactgctaccatggtgatggacagagctaccgaggcacatcctccaccaccaccacaggaaagaagtgtcagtcttggtcatctatgacaccacaccggcaccagaagaccccagaaaactacccaaatgctggcctgacaatgaactactgcaggaatccagatgccgataaaggcccctggtgttttaccacagaccccagcgtcaggtgggagtactgcaacctgaaaaaatgctcaggaacagaagcgagtgttgtagcacctccgcctgttgtcctgcttccagatgtagagactccttccgaagaagactgtatgtttgggaatgggaaaggataccgaggcaagagggcgaccactgttactgggacgccatgccaggactgggctgcccaggagccccatagacacagcattttcactccagagacaaatccacgggcgggtctggaaaaaaattactgccgtaaccctgatggtgatgtaggtggtccctggtgctacacgacaaatccaagaaaactttacgactactgtgatgtccctcagtgtgcggccccttcatttgattgtgggaagcctcaagtggagccgaagaaatgtcctggaagggttgtaggggggtgtgtggcccacccacattcctggccctggcaagtcagtcttagaacaaggtttggaatgcacttctgtggaggcaccttgatatccccagagtgggtgttgactgctgcccactgcttggagaagtccccaaggccttcatcctacaaggtcatcctgggtgcacaccaagaagtgaatctcgaaccgcatgttcaggaaatagaagtgtctaggctgttcttggagcccacacgaaaagatattgccttgctaaagctaagcagtcctgccgtcatcactgacaaagtaatcccagcttgtctgccatccccaaattatgtggtcgctgaccggaccgaatgtttcatcactggctggggagaaacccaaggtacttttggagctggccttctcaaggaagcccagctccctgtgattgagaataaagtgtgcaatcgctatgagtttctgaatggaagagtccaatccaccgaactctgtgctgggcatttggccggaggcactgacagttgccagggtgacagtggaggtcctctggtttgcttcgagaaggacaaatacattttacaaggagtcacttcttggggtcttggctgtgcacgccccaataagcctggtgtctatgttcgtgtttcaaggtttgttacttggattgagggagtgatgagaaataattaa

SEQ ID NO: 4 - protein, 810 aa, Artificial sequence
  amino acid sequence of the natural plasminogen(from swiss prot)with the signal peptide
MEHKEVVLLLLLFLKSGQGEPLDDYVNTQGASLFSVTKKQLGAGSIEECAAKCEEDEEFTCRAFQYHSKEQQCVIMAENRKSSIIIRMRDVVLFEKKVYLSECKTGNGKNYRGTMSKTKNGITCQKWSSTSPHRPRFSPATHPSEGLEENYCRNPDNDPQGPWCYTTDPEKRYDYCDILECEEECMHCSGENYDGKISKTMSGLECQAWDSQSPHAHGYIPSKFPNKNLKKNYCRNPDRELRPWCFTTDPNKRWELCDIPRCTTPPPSSGPTYQCLKGTGENYRGNVAVTVSGHTCQHWSAQTPHTHNRTPENFPCKNLDENYCRNPDGKRAPWCHTTNSQVRWEYCKIPSCDSSPVSTEQLAPTAPPELTPVVQDCYHGDGQSYRGTSSTTTTGKKCQSWSSMTPHRHQKTPENYPNAGLTMNYCRNPDADKGPWCFTTDPSVRWEYCNLKKCSGTEASVVAPPPVVLLPDVETPSEEDCMFGNGKGYRGKRATTVTGTPCQDWAAQEPHRHSIFTPETNPRAGLEKNYCRNPDGDVGGPWCYTTNPRKLYDYCDVPQCAAPSFDCGKPQVEPKKCPGRVVGGCVAHPHSWPWQVSLRTRFGMHFCGGTLISPEWVLTAAHCLEKSPRPSSYKVILGAHQEVNLEPHVQEIEVSRLFLEPTRKDIALLKLSSPAVITDKVIPACLPSPNYVVADRTECFITGWGETQGTFGAGLLKEAQLPVIENKVCNRYEFLNGRVQSTELCAGHLAGGTDSCQGDSGGPLVCFEKDKYILQGVTSWGLGCARPNKPGVYVRVSRFVTWIEGVMRNN

SEQ ID NO: 5 - DNA, 2145 bp, Artificial sequence
  nucleotide sequence of LYS77-PLG(Lys-plasminogen)
aaagtgtatctctcagagtgcaagactgggaatggaaagaactacagagggacgatgtccaaaacaaaaaatggcatcacctgtcaaaaatggagttccacttctccccacagacctagattctcacctgctacacacccctcagagggactggaggagaactactgcaggaatccagacaacgatccgcaggggccctggtgctatactactgatccagaaaagagatatgactactgcgacattcttgagtgtgaagaggaatgtatgcattgcagtggagaaaactatgacggcaaaatttccaagaccatgtctggactggaatgccaggcctgggactctcagagcccacacgctcatggatacattccttccaaatttccaaacaagaacctgaagaagaattactgtcgtaaccccgatagggagctgcggccttggtgtttcaccaccgaccccaacaagcgctgggaactttgtgacatcccccgctgcacaacacctccaccatcttctggtcccacctaccagtgtctgaagggaacaggtgaaaactatcgcgggaatgtggctgttaccgtgtccgggcacacctgtcagcactggagtgcacagacccctcacacacataacaggacaccagaaaacttcccctgcaaaaatttggatgaaaactactgccgcaatcctgacggaaaaagggccccatggtgccatacaaccaacagccaagtgcggtgggagtactgtaagataccgtcctgtgactcctccccagtatccacggaacaattggctcccacagcaccacctgagctaacccctgtggtccaggactgctaccatggtgatggacagagctaccgaggcacatcctccaccaccaccacaggaaagaagtgtcagtcttggtcatctatgacaccacaccggcaccagaagaccccagaaaactacccaaatgctggcctgacaatgaactactgcaggaatccagatgccgataaaggcccctggtgttttaccacagaccccagcgtcaggtgggagtactgcaacctgaaaaaatgctcaggaacagaagcgagtgttgtagcacctccgcctgttgtcctgcttccagatgtagagactccttccgaagaagactgtatgtttgggaatgggaaaggataccgaggcaagagggcgaccactgttactgggacgccatgccaggactgggctgcccaggagccccatagacacagcattttcactccagagacaaatccacgggcgggtctggaaaaaaattactgccgtaaccctgatggtgatgtaggtggtccctggtgctacacgacaaatccaagaaaactttacgactactgtgatgtccctcagtgtgcggccccttcatttgattgtgggaagcctcaagtggagccgaagaaatgtcctggaagggttgtaggggggtgtgtggcccacccacattcctggccctggcaagtcagtcttagaacaaggtttggaatgcacttctgtggaggcaccttgatatccccagagtgggtgttgactgctgcccactgcttggagaagtccccaaggccttcatcctacaaggtcatcctgggtgcacaccaagaagtgaatctcgaaccgcatgttcaggaaatagaagtgtctaggctgttcttggagcccacacgaaaagatattgccttgctaaagctaagcagtcctgccgtcatcactgacaaagtaatcccagcttgtctgccatccccaaattatgtggtcgctgaccggaccgaatgtttcatcactggctggggagaaacccaaggtacttttggagctggccttctcaaggaagcccagctccctgtgattgagaataaagtgtgcaatcgctatgagtttctgaatggaagagtccaatccaccgaactctgtgctgggcatttggccggaggcactgacagttgccagggtgacagtggaggtcctctggtttgcttcgagaaggacaaatacattttacaaggagtcacttcttggggtcttggctgtgcacgccccaataagcctggtgtctatgttcgtgtttcaaggtttgttacttggattgagggagtgatgagaaataattaa

SEQ ID NO: 6 - protein, 714 aa, Artificial sequence
  amino acid sequence of LYS77-PLG(Lys-plasminogen)
KVYLSECKTGNGKNYRGTMSKTKNGITCQKWSSTSPHRPRFSPATHPSEGLEENYCRNPDNDPQGPWCYTTDPEKRYDYCDILECEEECMHCSGENYDGKISKTMSGLECQAWDSQSPHAHGYIPSKFPNKNLKKNYCRNPDRELRPWCFTTDPNKRWELCDIPRCTTPPPSSGPTYQCLKGTGENYRGNVAVTVSGHTCQHWSAQTPHTHNRTPENFPCKNLDENYCRNPDGKRAPWCHTTNSQVRWEYCKIPSCDSSPVSTEQLAPTAPPELTPVVQDCYHGDGQSYRGTSSTTTTGKKCQSWSSMTPHRHQKTPENYPNAGLTMNYCRNPDADKGPWCFTTDPSVRWEYCNLKKCSGTEASVVAPPPVVLLPDVETPSEEDCMFGNGKGYRGKRATTVTGTPCQDWAAQEPHRHSIFTPETNPRAGLEKNYCRNPDGDVGGPWCYTTNPRKLYDYCDVPQCAAPSFDCGKPQVEPKKCPGRVVGGCVAHPHSWPWQVSLRTRFGMHFCGGTLISPEWVLTAAHCLEKSPRPSSYKVILGAHQEVNLEPHVQEIEVSRLFLEPTRKDIALLKLSSPAVITDKVIPACLPSPNYVVADRTECFITGWGETQGTFGAGLLKEAQLPVIENKVCNRYEFLNGRVQSTELCAGHLAGGTDSCQGDSGGPLVCFEKDKYILQGVTSWGLGCARPNKPGVYVRVSRFVTWIEGVMRNN

SEQ ID NO: 7 - DNA, 1245 bp, Artificial sequence
  nucleotide sequence of delta-plg(delta-plasminogen)
gagcctctggatgactatgtgaatacccagggggcttcactgttcagtgtcactaagaagcagctgggagcaggaagtatagaagaatgtgcagcaaaatgtgaggaggacgaagaattcacctgcagggcattccaatatcacagtaaagagcaacaatgtgtgataatggctgaaaacaggaagtcctccataatcattaggatgagagatgtagttttatttgaaaagaaagtgtatctctcagagtgcaagactgggaatggaaagaactacagagggacgatgtccaaaacaaaaaatggcatcacctgtcaaaaatggagttccacttctccccacagacctagattctcacctgctacacacccctcagagggactggaggagaactactgcaggaatccagacaacgatccgcaggggccctggtgctatactactgatccagaaaagagatatgactactgcgacattcttgagtgtgaagaggcggccccttcatttgattgtgggaagcctcaagtggagccgaagaaatgtcctggaagggttgtaggggggtgtgtggcccacccacattcctggccctggcaagtcagtcttagaacaaggtttggaatgcacttctgtggaggcaccttgatatccccagagtgggtgttgactgctgcccactgcttggagaagtccccaaggccttcatcctacaaggtcatcctgggtgcacaccaagaagtgaatctcgaaccgcatgttcaggaaatagaagtgtctaggctgttcttggagcccacacgaaaagatattgccttgctaaagctaagcagtcctgccgtcatcactgacaaagtaatcccagcttgtctgccatccccaaattatgtggtcgctgaccggaccgaatgtttcatcactggctggggagaaacccaaggtacttttggagctggccttctcaaggaagcccagctccctgtgattgagaataaagtgtgcaatcgctatgagtttctgaatggaagagtccaatccaccgaactctgtgctgggcatttggccggaggcactgacagttgccagggtgacagtggaggtcctctggtttgcttcgagaaggacaaatacattttacaaggagtcacttcttggggtcttggctgtgcacgccccaataagcctggtgtctatgttcgtgtttcaaggtttgttacttggattgagggagtgatgagaaataattaa

SEQ ID NO: 8 - protein, 414 aa, Artificial sequence
  amino acid sequence of delta-plg(delta-plasminogen)
EPLDDYVNTQGASLFSVTKKQLGAGSIEECAAKCEEDEEFTCRAFQYHSKEQQCVIMAENRKSSIIIRMRDVVLFEKKVYLSECKTGNGKNYRGTMSKTKNGITCQKWSSTSPHRPRFSPATHPSEGLEENYCRNPDNDPQGPWCYTTDPEKRYDYCDILECEEAAPSFDCGKPQVEPKKCPGRVVGGCVAHPHSWPWQVSLRTRFGMHFCGGTLISPEWVLTAAHCLEKSPRPSSYKVILGAHQEVNLEPHVQEIEVSRLFLEPTRKDIALLKLSSPAVITDKVIPACLPSPNYVVADRTECFITGWGETQGTFGAGLLKEAQLPVIENKVCNRYEFLNGRVQSTELCAGHLAGGTDSCQGDSGGPLVCFEKDKYILQGVTSWGLGCARPNKPGVYVRVSRFVTWIEGVMRNN

SEQ ID NO: 9 - DNA, 1104 bp, Artificial sequence
  nucleotide sequence of Mini-plg(mini-plasminogen)
gtcaggtgggagtactgcaacctgaaaaaatgctcaggaacagaagcgagtgttgtagcacctccgcctgttgtcctgcttccagatgtagagactccttccgaagaagactgtatgtttgggaatgggaaaggataccgaggcaagagggcgaccactgttactgggacgccatgccaggactgggctgcccaggagccccatagacacagcattttcactccagagacaaatccacgggcgggtctggaaaaaaattactgccgtaaccctgatggtgatgtaggtggtccctggtgctacacgacaaatccaagaaaactttacgactactgtgatgtccctcagtgtgcggccccttcatttgattgtgggaagcctcaagtggagccgaagaaatgtcctggaagggttgtaggggggtgtgtggcccacccacattcctggccctggcaagtcagtcttagaacaaggtttggaatgcacttctgtggaggcaccttgatatccccagagtgggtgttgactgctgcccactgcttggagaagtccccaaggccttcatcctacaaggtcatcctgggtgcacaccaagaagtgaatctcgaaccgcatgttcaggaaatagaagtgtctaggctgttcttggagcccacacgaaaagatattgccttgctaaagctaagcagtcctgccgtcatcactgacaaagtaatcccagcttgtctgccatccccaaattatgtggtcgctgaccggaccgaatgtttcatcactggctggggagaaacccaaggtacttttggagctggccttctcaaggaagcccagctccctgtgattgagaataaagtgtgcaatcgctatgagtttctgaatggaagagtccaatccaccgaactctgtgctgggcatttggccggaggcactgacagttgccagggtgacagtggaggtcctctggtttgcttcgagaaggacaaatacattttacaaggagtcacttcttggggtcttggctgtgcacgccccaataagcctggtgtctatgttcgtgtttcaaggtttgttacttggattgagggagtgatgagaaataattaa

SEQ ID NO: 10 - protein, 367 aa, Artificial sequence
  amino acid sequence of Mini-plg(mini-plasminogen)
VRWEYCNLKKCSGTEASVVAPPPVVLLPDVETPSEEDCMFGNGKGYRGKRATTVTGTPCQDWAAQEPHRHSIFTPETNPRAGLEKNYCRNPDGDVGGPWCYTTNPRKLYDYCDVPQCAAPSFDCGKPQVEPKKCPGRVVGGCVAHPHSWPWQVSLRTRFGMHFCGGTLISPEWVLTAAHCLEKSPRPSSYKVILGAHQEVNLEPHVQEIEVSRLFLEPTRKDIALLKLSSPAVITDKVIPACLPSPNYVVADRTECFITGWGETQGTFGAGLLKEAQLPVIENKVCNRYEFLNGRVQSTELCAGHLAGGTDSCQGDSGGPLVCFEKDKYILQGVTSWGLGCARPNKPGVYVRVSRFVTWIEGVMRNN

SEQ ID NO: 11 - DNA, 750 bp, Artificial sequence
  nucleotide sequence of Micro-plg(micro-plasminogen)
gccccttcatttgattgtgggaagcctcaagtggagccgaagaaatgtcctggaagggttgtaggggggtgtgtggcccacccacattcctggccctggcaagtcagtcttagaacaaggtttggaatgcacttctgtggaggcaccttgatatccccagagtgggtgttgactgctgcccactgcttggagaagtccccaaggccttcatcctacaaggtcatcctgggtgcacaccaagaagtgaatctcgaaccgcatgttcaggaaatagaagtgtctaggctgttcttggagcccacacgaaaagatattgccttgctaaagctaagcagtcctgccgtcatcactgacaaagtaatcccagcttgtctgccatccccaaattatgtggtcgctgaccggaccgaatgtttcatcactggctggggagaaacccaaggtacttttggagctggccttctcaaggaagcccagctccctgtgattgagaataaagtgtgcaatcgctatgagtttctgaatggaagagtccaatccaccgaactctgtgctgggcatttggccggaggcactgacagttgccagggtgacagtggaggtcctctggtttgcttcgagaaggacaaatacattttacaaggagtcacttcttggggtcttggctgtgcacgccccaataagcctggtgtctatgttcgtgtttcaaggtttgttacttggattgagggagtgatgagaaataattaa

SEQ ID NO: 12 - protein, 249 aa, Artificial sequence
  amino acid sequence of Micro-plg(micro-plasminogen)
APSFDCGKPQVEPKKCPGRVVGGCVAHPHSWPWQVSLRTRFGMHFCGGTLISPEWVLTAAHCLEKSPRPSSYKVILGAHQEVNLEPHVQEIEVSRLFLEPTRKDIALLKLSSPAVITDKVIPACLPSPNYVVADRTECFITGWGETQGTFGAGLLKEAQLPVIENKVCNRYEFLNGRVQSTELCAGHLAGGTDSCQGDSGGPLVCFEKDKYILQGVTSWGLGCARPNKPGVYVRVSRFVTWIEGVMRNN

SEQ ID NO: 13 - DNA, 684 bp, Artificial sequence
  nucleotide sequence of the serine protease domain
gttgtaggggggtgtgtggcccacccacattcctggccctggcaagtcagtcttagaacaaggtttggaatgcacttctgtggaggcaccttgatatccccagagtgggtgttgactgctgcccactgcttggagaagtccccaaggccttcatcctacaaggtcatcctgggtgcacaccaagaagtgaatctcgaaccgcatgttcaggaaatagaagtgtctaggctgttcttggagcccacacgaaaagatattgccttgctaaagctaagcagtcctgccgtcatcactgacaaagtaatcccagcttgtctgccatccccaaattatgtggtcgctgaccggaccgaatgtttcatcactggctggggagaaacccaaggtacttttggagctggccttctcaaggaagcccagctccctgtgattgagaataaagtgtgcaatcgctatgagtttctgaatggaagagtccaatccaccgaactctgtgctgggcatttggccggaggcactgacagttgccagggtgacagtggaggtcctctggtttgcttcgagaaggacaaatacattttacaaggagtcacttcttggggtcttggctgtgcacgccccaataagcctggtgtctatgttcgtgtttcaaggtttgttacttggattgagggagtgatgaga

SEQ ID NO: 14 - protein, 228 aa, Artificial sequence
  amino acid sequence of the serine protease domain
VVGGCVAHPHSWPWQVSLRTRFGMHFCGGTLISPEWVLTAAHCLEKSPRPSSYKVILGAHQEVNLEPHVQEIEVSRLFLEPTRKDIALLKLSSPAVITDKVIPACLPSPNYVVADRTECFITGWGETQGTFGAGLLKEAQLPVIENKVCNRYEFLNGRVQSTELCAGHLAGGTDSCQGDSGGPLVCFEKDKYILQGVTSWGLGCARPNKPGVYVRVSRFVTWIEGVMR